European Patent Application EP 4 458 968 A1, published November 6, 2024. Title: Circular nucleic acids and uses thereof for shaping the cellular proteome. Applicant: Justus-Liebig-Universität Gießen. The sequence listing filed with the application follows.

SEQUENCE LISTING (74 sequences)

SEQ ID NO: 1 - RNA, 164 nt, Homo sapiens
  source 1..164: mol_type = other RNA
atacttacctggcaggggagataccatgatcacgaaggtggttttcccagggcgaggcttatccattgcactccggatgtgctgacccctgcgatttccccaaatgtgggaaactcgactgcataatttgtggtagtgggggactgcgttcgcgctttcccctg

SEQ ID NO: 2 - DNA, 11 bp, synthetic construct
  source 1..11: mol_type = other DNA
caggtaagtat

SEQ ID NO: 3 - DNA, 20 bp, synthetic construct
  source 1..20: mol_type = other DNA
ctcccctgccaggtaagtat

SEQ ID NO: 4 - DNA, 22 bp, synthetic construct
  source 1..22: mol_type = other DNA
atctcccctgccaggtaagtat

SEQ ID NO: 5 - DNA, 30 bp, synthetic construct
  source 1..30: mol_type = other DNA
atcatggtatctcccctgccaggtaagtat

SEQ ID NO: 6 - DNA, 42 bp, synthetic construct
  source 1..42: mol_type = other DNA
accaccttcgtgatcatggtatctcccctgccaggtaagtat

SEQ ID NO: 7 - DNA, 83 bp, synthetic construct
  source 1..83: mol_type = other DNA
ggtatctcccctgccaggtaagtatatatggtatctcccctgccaggtaagtatatatggtatctcccctgccaggtaagtat

SEQ ID NO: 8 - DNA, 66 bp, synthetic construct
  source 1..66: mol_type = other DNA
atcatggtatctcccctgccaggtaagtataattaaatcatggtatctcccctgccaggtaagtat

SEQ ID NO: 9 - DNA, 102 bp, synthetic construct
  source 1..102: mol_type = other DNA
atcatggtatctcccctgccaggtaagtataattaaatcatggtatctcccctgccaggtaagtataattaaatcatggtatctcccctgccaggtaagtat

SEQ ID NO: 10 - RNA, 324 nt, Homo sapiens
  source 1..324: mol_type = mRNA
gtagggggcgcgcaccgaggcaccgcggcgagcttggctgcttctggggcctgtgtggccctgtgtgtcggaaagatggagcaagaagccgagcccgaggggcggccgcgacccctctgaccgagatcctgctgctttcgcagccaggagcaccgtccctccccggattagtgcgtacgagcgcccagtgccctggcccggagagtggaatgatccccgaggcccagggcgtcgtgcttccgcgcgccccgtgaaggaaactggggagtcttgagggacccccgactccaagcgcgaaaaccccggatggtgaggagcaggcaa

SEQ ID NO: 11 - DNA, 19 bp, synthetic construct
  source 1..19: mol_type = other DNA
cagccaagctcgccgcggt

SEQ ID NO: 12 - DNA, 31 bp, synthetic construct
  source 1..31: mol_type = other DNA
cagccaagctcgccgcggtgcctcggtgcgc

SEQ ID NO: 13 - DNA, 40 bp, synthetic construct
  source 1..40: mol_type = other DNA
cagccaagctcgccgcggtgcctcggtgcgcgccccctac

SEQ ID NO: 14 - DNA, 29 bp, synthetic construct
  source 1..29: mol_type = other DNA
gccccagaagcagccaagctcgccgcggt

SEQ ID NO: 15 - DNA, 39 bp, synthetic construct
  source 1..39: mol_type = other DNA
ggccacacaggccccagaagcagccaagctcgccgcggt

SEQ ID NO: 16 - DNA, 20 bp, synthetic construct
  source 1..20: mol_type = other DNA
  misc_difference 3: replace = a; replace = c; replace = g; replace = t
tcntgctccatctttccgac

SEQ ID NO: 17 - DNA, 30 bp, synthetic construct
  source 1..30: mol_type = other DNA
  misc_difference 3: replace = a; replace = c; replace = g; replace = t
tcntgctccatctttccgacacacagggcc

SEQ ID NO: 18 - DNA, 40 bp, synthetic construct
  source 1..40: mol_type = other DNA
  misc_difference 3: replace = a; replace = c; replace = g; replace = t
tcntgctccatctttccgacacacagggccacacaggccc

SEQ ID NO: 19 - DNA, 30 bp, synthetic construct
  source 1..30: mol_type = other DNA
  misc_difference 13: replace = a; replace = c; replace = g; replace = t
gggctcggcttcntgctccatctttccgac

SEQ ID NO: 20 - DNA, 40 bp, synthetic construct
  source 1..40: mol_type = other DNA
  misc_difference 23: replace = a; replace = c; replace = g; replace = t
gccgcccctcgggctcggcttcntgctccatctttccgac

SEQ ID NO: 21 - DNA, 40 bp, synthetic construct
  source 1..40: mol_type = other DNA
  misc_difference 13: replace = a; replace = c; replace = g; replace = t
gggctcggcttcntgctccatctttccgacacacagggcc

SEQ ID NO: 22 - DNA, 20 bp, synthetic construct
  source 1..20: mol_type = other DNA
gacggtgctcctggctgcga

SEQ ID NO: 23 - DNA, 30 bp, synthetic construct
  source 1..30: mol_type = other DNA
gacggtgctcctggctgcgaaagcagcagg

SEQ ID NO: 24 - DNA, 40 bp, synthetic construct
  source 1..40: mol_type = other DNA
gacggtgctcctggctgcgaaagcagcaggatctcggtca

SEQ ID NO: 25 - DNA, 30 bp, synthetic construct
  source 1..30: mol_type = other DNA
tccggggagggacggtgctcctggctgcga

SEQ ID NO: 26 - DNA, 40 bp, synthetic construct
  source 1..40: mol_type = other DNA
tacgcactaatccggggagggacggtgctcctggctgcga

SEQ ID NO: 27 - DNA, 40 bp, synthetic construct
  source 1..40: mol_type = other DNA
tccggggagggacggtgctcctggctgcgaaagcagcagg

SEQ ID NO: 28 - DNA, 18 bp, synthetic construct
  source 1..18: mol_type = other DNA
gctcctcaccatccgggg

SEQ ID NO: 29 - DNA, 40 bp, synthetic construct
  source 1..40: mol_type = other DNA
  misc_difference 21: replace = a; replace = c; replace = g; replace = t
gctcctcaccatccggggttntcgcgcttggagtcggggg

SEQ ID NO: 30 - DNA, 50 bp, synthetic construct
  source 1..50: mol_type = other DNA
  misc_difference 21: replace = a; replace = c; replace = g; replace = t
gctcctcaccatccggggttntcgcgcttggagtcgggggtccctcaaga

SEQ ID NO: 31 - DNA, 24 bp, synthetic construct
  source 1..24: mol_type = other DNA
ttgcctgctcctcaccatccgggg

SEQ ID NO: 32 - RNA, 67 nt, Homo sapiens
  source 1..67: mol_type = mRNA
agtggcgattggagggtagacctgtgggcacggacgcacgccactttttctctgctgatccaggcaa

SEQ ID NO: 33 - DNA, 19 bp, synthetic construct
  source 1..19: mol_type = other DNA
cgtgcgtccgtgcccacag

SEQ ID NO: 34 - DNA, 31 bp, synthetic construct
  source 1..31: mol_type = other DNA
cgtgcgtccgtgcccacaggtctaccctcca

SEQ ID NO: 35 - DNA, 40 bp, synthetic construct
  source 1..40: mol_type = other DNA
cgtgcgtccgtgcccacaggtctaccctccaatcgccact

SEQ ID NO: 36 - DNA, 29 bp, synthetic construct
  source 1..29: mol_type = other DNA
gaaaaagtggcgtgcgtccgtgcccacag

SEQ ID NO: 37 - DNA, 40 bp, synthetic construct
  source 1..40: mol_type = other DNA
ggatcagcagagaaaaagtggcgtgcgtccgtgcccacag

SEQ ID NO: 38 - DNA, 24 bp, synthetic construct
  source 1..24: mol_type = other DNA
ttgcctggatcagcagagaaaaag

SEQ ID NO: 39 - DNA, 34 bp, synthetic construct
  source 1..34: mol_type = other DNA
ttgcctggatcagcagagaaaaagaccgcacgca

SEQ ID NO: 40 - RNA, 50 nt, Homo sapiens
  source 1..50: mol_type = mRNA
acatttgcttctgacacaactgtgttcactagcaacctcaaacagacacc

SEQ ID NO: 41 - DNA, 28 bp, synthetic construct
  source 1..28: mol_type = other DNA
tgtttgaggttgctagtgaacacagttg

SEQ ID NO: 42 - DNA, 35 bp, synthetic construct
  source 1..35: mol_type = other DNA
tgtttgaggttgctagtgaacacagttgtgtcaga

SEQ ID NO: 43 - DNA, 44 bp, synthetic construct
  source 1..44: mol_type = other DNA
tgtttgaggttgctagtgaacacagttgtgtcagaagcaaatgt

SEQ ID NO: 44 - DNA, 34 bp, synthetic construct
  source 1..34: mol_type = other DNA
ggtgtctgtttgaggttgctagtgaacacagttg

SEQ ID NO: 45 - DNA, 42 bp, synthetic construct
  source 1..42: mol_type = other DNA
tgtttgaggttgctagtgaacacagttgtgtcagaagcaaat

SEQ ID NO: 46 - DNA, 31 bp, synthetic construct
  source 1..31: mol_type = other DNA
tgtttgaggttgctagtgaacacagttgtgt

SEQ ID NO: 47 - DNA, 31 bp, synthetic construct
  source 1..31: mol_type = other DNA
gtctgtttgaggttgctagtgaacacagttg

SEQ ID NO: 48 - DNA, 31 bp, synthetic construct
  source 1..31: mol_type = other DNA
gggagtaagccaggtaagtatgcttacagta

SEQ ID NO: 49 - DNA, 42 bp, synthetic construct
  source 1..42: mol_type = other DNA
gggagtaagcatctcccctgccaggtaagtatgcttacagta

SEQ ID NO: 50 - DNA, 50 bp, synthetic construct
  source 1..50: mol_type = other DNA
gggagtaagcatcatggtatctcccctgccaggtaagtatgcttacagta

SEQ ID NO: 51 - DNA, 62 bp, synthetic construct
  source 1..62: mol_type = other DNA
gggagtaagcaccaccttcgtgatcatggtatctcccctgccaggtaagtatgcttacagta

SEQ ID NO: 52 - DNA, 86 bp, synthetic construct
  source 1..86: mol_type = other DNA
gggagtaagcatcatggtatctcccctgccaggtaagtataattaaatcatggtatctcccctgccaggtaagtatgcttacagta

SEQ ID NO: 53 - DNA, 103 bp, synthetic construct
  source 1..103: mol_type = other DNA
gggagtaagcggtatctcccctgccaggtaagtatatatggtatctcccctgccaggtaagtatatatggtatctcccctgccaggtaagtatgcttacagta

SEQ ID NO: 54 - DNA, 40 bp, synthetic construct
  source 1..40: mol_type = other DNA
gggagtaagccctgcctgtctattgatgtcgcttacagta

SEQ ID NO: 55 - DNA, 62 bp, synthetic construct
  source 1..62: mol_type = other DNA
gggagtaagctgtttgaggttgctagtgaacacagttgtgtcagaagcaaatgcttacagta

SEQ ID NO: 56 - DNA, 51 bp, synthetic construct
  source 1..51: mol_type = other DNA
gggagtaagctgtttgaggttgctagtgaacacagttgtgtgcttacagta

SEQ ID NO: 57 - DNA, 51 bp, synthetic construct
  source 1..51: mol_type = other DNA
gggagtaagcgtctgtttgaggttgctagtgaacacagttggcttacagta

SEQ ID NO: 58 - DNA, 61 bp, synthetic construct
  source 1..61: mol_type = other DNA
gggagtaagcgggcctttctttatgtttttggcgtcggatcccatggtgtcgcttacagta

SEQ ID NO: 59 - DNA, 50 bp, synthetic construct
  source 1..50: mol_type = other DNA
gggagtaagcggaaccagggcgtatctcttcatagccttagcttacagta

SEQ ID NO: 60 - DNA, 45 bp, synthetic construct
  source 1..45: mol_type = other DNA
gggagtaagcagatgcgcaccgcacagatgcgcacgcttacagta

SEQ ID NO: 61 - DNA, 90 bp, synthetic construct
  source 1..90: mol_type = other DNA
aaccatgccgagtgcggccgcaacagccaagctcgccgcggtgcctcggtgcgcgccccctacaaaaaccgcggtcggcgtggactgtag

SEQ ID NO: 62 - DNA, 90 bp, synthetic construct
  source 1..90: mol_type = other DNA
aaccatgccgagtgcggccgcaagggctcggcttcatgctccatctttccgacacacagggccaaaaaccgcggtcggcgtggactgtag

SEQ ID NO: 63 - DNA, 90 bp, synthetic construct
  source 1..90: mol_type = other DNA
aaccatgccgagtgcggccgcaatccggggagggacggtgctcctggctgcgaaagcagcaggaaaaaccgcggtcggcgtggactgtag

SEQ ID NO: 64 - DNA, 90 bp, synthetic construct
  source 1..90: mol_type = other DNA
aaccatgccgagtgcggccgcaaccctgggcctcggggatcattccactctccgggccagggcaaaaaccgcggtcggcgtggactgtag

SEQ ID NO: 65 - DNA, 90 bp, synthetic construct
  source 1..90: mol_type = other DNA
aaccatgccgagtgcggccgcaaggagtcgggggtccctcaagactccccagtatccttcacgaaaaaccgcggtcggcgtggactgtag

SEQ ID NO: 66 - DNA, 90 bp, synthetic construct
  source 1..90: mol_type = other DNA
aaccatgccgagtgcggccgcaagctcctcaccatccggggttatcgcgcttggagtcgggggaaaaaccgcggtcggcgtggactgtag

SEQ ID NO: 67 - DNA, 90 bp, synthetic construct
  source 1..90: mol_type = other DNA
aaccatgccgagtgcggccgcaatgttggtattgcacatttgcctgctcctcaccatccggggaaaaaccgcggtcggcgtggactgtag

SEQ ID NO: 68 - DNA, 90 bp, synthetic construct
  source 1..90: mol_type = other DNA
aaccatgccgagtgcggccgcaacgtgcgtccgtgcccacaggtctaccctccaatcgccactaaaaaccgcggtcggcgtggactgtag

SEQ ID NO: 69 - DNA, 90 bp, synthetic construct
  source 1..90: mol_type = other DNA
aaccatgccgagtgcggccgcaaggatcagcagagaaaaagtggcgtgcgtccgtgcccacagaaaaaccgcggtcggcgtggactgtag

SEQ ID NO: 70 - DNA, 90 bp, synthetic construct
  source 1..90: mol_type = other DNA
aaccatgccgagtgcggccgcaatgttggtattgcacatttgcctggatcagcagagaaaaagaaaaaccgcggtcggcgtggactgtag

SEQ ID NO: 71 - DNA, 90 bp, synthetic construct
  source 1..90: mol_type = other DNA
aaccatgccgagtgcggccgcaaagatgcgcaccgcacagatgcgcaccacgccacgcgtagaaaaaaccgcggtcggcgtggactgtag

SEQ ID NO: 72 - DNA, 90 bp, synthetic construct
  source 1..90: mol_type = other DNA
aaccatgccgagtgcggccgcaaagtcagtgagtcagtgtaatacgggaggatacccgctgtcaaaaaccgcggtcggcgtggactgtag

SEQ ID NO: 73 - RNA, 324 nt, synthetic construct
  source 1..324: mol_type = other RNA
gtagggggcgcgcaccgaggcaccgcggcgagcttggctgcttctggggcctgtgtggccctgtgtgtcggaaagaaggagcaagaagccgagcccgaggggcggccgcgacccctctgaccgagatcctgctgctttcgcagccaggagcaccgtccctccccggattagtgcgtacgagcgcccagtgccctggcccggagagtggaaagatccccgaggcccagggcgtcgtgcttccgcgcgccccgtgaaggaaactggggagtcttgagggacccccgactccaagcgcgaaaaccccggatggtgaggagcaggcaa

SEQ ID NO: 74 - RNA, 47 nt, Homo sapiens
  source 1..47: mol_type = other RNA
atacttacctggcaggggagataccatgatcacgaaggtggttttcc